European Patent Application EP 4 309 677 A1, published January 24, 2024. Title: PD-L1 and TLR7 double-targeting nanobody coupling drug and use thereof in anti-tumor. Applicant: SHANGHAI INSTITUTE OF MATERIA MEDICA,CHINESE ACADEMY OF SCIENCES. Application PCT/CN2022/080953. The sequence listing filed with the application follows.

SEQUENCE LISTING (117 sequences)

SEQ ID NO: 1 - protein, 122 aa, Artificial Sequence
  Nb16 Amino acid sequence of VHH
QVQLQESGGGSVQAGGSLRLSCAASGYTDRNYWMGWFRQAPGKEREGVAALYTRTGSTYYADSVKGRFTISHDNAKNTLYLQMNSLKPEDTAVYYCAADSNAYGLAPLHHYWGQGTQVTVSS

SEQ ID NO: 2 - protein, 8 aa, Artificial Sequence
  Nb16 CDR1
GYTDRNYW

SEQ ID NO: 3 - protein, 8 aa, Artificial Sequence
  Nb16 CDR2
LYTRTGST

SEQ ID NO: 4 - protein, 15 aa, Artificial Sequence
  Nb16 CDR3
AADSNAYGLAPLHHY

SEQ ID NO: 5 - protein, 121 aa, Artificial Sequence
  Nb9 Amino acid sequence of VHH
QVQLQESGGGLVHPGGSLRLSCAASGFTFSSYTMRWVRQAPGKGLEWVSGINNVGGSTLYADSVKGRFTISRDNAKNTLYLQMNSLQPDDTAMYYCATGIIGSGLETATYRGQGTQVTVSS

SEQ ID NO: 6 - protein, 8 aa, Artificial Sequence
  Nb9 CDR1
GFTFSSYT

SEQ ID NO: 7 - protein, 8 aa, Artificial Sequence
  Nb9 CDR2
INNVGGST

SEQ ID NO: 8 - protein, 12 aa, Artificial Sequence
  Nb9 CDR3
ATGIIGSGLETA

SEQ ID NO: 9 - protein, 122 aa, Artificial Sequence
  Nb10 Amino acid sequence of VHH
QVQLQESGGGSVQAGGSLRLSCAASGYRFCRLAMRWYRQAPGKEREFVSFIDSGGTTSYADSVKGRFTISRDSAKNTVYLQMNSLKPEDTGMYYCNSDILGGGGGCPVSSYWGQGTQVTVSS

SEQ ID NO: 10 - protein, 8 aa, Artificial Sequence
  Nb10 CDR1
GYRFCRLA

SEQ ID NO: 11 - protein, 7 aa, Artificial Sequence
  Nb10 CDR2
IDSGGTT

SEQ ID NO: 12 - protein, 16 aa, Artificial Sequence
  Nb10 CDR3
NSDILGGGGGCPVSSY

SEQ ID NO: 13 - protein, 126 aa, Artificial Sequence
  Nb11 Amino acid sequence of VHH
QVQLQESGGGSVQAEGSLRLSCSAPIYVTYYGTYCMGWFRQAPGKEREGVAGISGDGRTSYADSVKGRFTVSKDNAKNTLYLEMNSLKPEDTAMYYCALRIGGYCDTLNGADFRYWGQGTQVTVSS

SEQ ID NO: 14 - protein, 10 aa, Artificial Sequence
  Nb11 CDR1
IYVTYYGTYC

SEQ ID NO: 15 - protein, 7 aa, Artificial Sequence
  Nb11 CDR2
ISGDGRT

SEQ ID NO: 16 - protein, 18 aa, Artificial Sequence
  Nb11 CDR3
ALRIGGYCDTLNGADFRY

SEQ ID NO: 17 - protein, 125 aa, Artificial Sequence
  Nb17 Amino acid sequence of VHH
QVQLQESGGGSVQAGGSLRLSCAASGYSARRRMGWFRQAPGKEREGVASIYTAGGRTWYADSVKGRFTISQDNAKNTVYLQMNSLKPDDTAMYYCAASPAPYGAESLSEADFAYWGQGTQVTVSS

SEQ ID NO: 18 - protein, 7 aa, Artificial Sequence
  Nb17 CDR1
GYSARRR

SEQ ID NO: 19 - protein, 7 aa, Artificial Sequence
  Nb17 CDR2
IYTAGGR

SEQ ID NO: 20 - protein, 19 aa, Artificial Sequence
  Nb17 CDR3
AASPAPYGAESLSEADFAY

SEQ ID NO: 21 - protein, 117 aa, Artificial Sequence
  h_Nb1 Amino acid sequence of VHH
DVQLQESGGGLVQPGGSLRLSCAASGFTFSSYAMSWVRQAPGKGLEWVSDINSGGDNTDYADSVKGRFTISRDNAKNTLYLQMNSLKPEDTAVYYCARGPKLCFSSWGQGTQVTVSS

SEQ ID NO: 22 - protein, 8 aa, Artificial Sequence
  h_Nb1CDR1,h_Nb6 CDR1
GFTFSSYA

SEQ ID NO: 23 - protein, 8 aa, Artificial Sequence
  h_Nb1 CDR2
INSGGDNT

SEQ ID NO: 24 - protein, 10 aa, Artificial Sequence
  h_Nb1 CDR3
ARGPKLCFSS

SEQ ID NO: 25 - protein, 115 aa, Artificial Sequence
  h_Nb2 Amino acid sequence of VHH
DVQLQESGGGLVQPGGSLRLSCAASGFTFGDRWMYWLRQAPGKGLEWVSSINPAGRSTYYADSVKGRFTISRDNAKNTLYLQMNSLKSEDTAVYYCTKDPGGYQKGQGTQVTVSS

SEQ ID NO: 26 - protein, 8 aa, Artificial Sequence
  h_Nb2 CDR1
GFTFGDRW

SEQ ID NO: 27 - protein, 8 aa, Artificial Sequence
  h_Nb2 CDR2
INPAGRST

SEQ ID NO: 28 - protein, 8 aa, Artificial Sequence
  h_Nb2 CDR3
TKDPGGYQ

SEQ ID NO: 29 - protein, 118 aa, Artificial Sequence
  h_Nb4 Amino acid sequence of VHH
DVQLQESGGGLVQAGGSLRLSCAAPSRMFSGYTMGWYRQAPGKQRELVAQIANGGFTDYIDSVKGRFSISRDTVLNMMYLQMNSLKPEDTAVYYCNLVLVNGIPTRNWGQGTQVTVSS

SEQ ID NO: 30 - protein, 8 aa, Artificial Sequence
  h_Nb4 CDR1
SRMFSGYT

SEQ ID NO: 31 - protein, 7 aa, Artificial Sequence
  h_Nb4 CDR2
IANGGFT

SEQ ID NO: 32 - protein, 12 aa, Artificial Sequence
  h_Nb4 CDR3
NLVLVNGIPTRN

SEQ ID NO: 33 - protein, 127 aa, Artificial Sequence
  h_Nb5 Amino acid sequence of VHH
DVQLQESGGGAVQSGESLRLSCAASGRDLMFYDVAWFRQAPGKEREGVSYIRSSGTLTKYADSVKGRFTISRDNDKNTVSLQMNSLNPEDTAKYYCAARLQSATSHSDLREDEFNSWGQGTQVTVSS

SEQ ID NO: 34 - protein, 8 aa, Artificial Sequence
  h_Nb5 CDR1
GRDLMFYD

SEQ ID NO: 35 - protein, 8 aa, Artificial Sequence
  h_Nb5 CDR2
IRSSGTLT

SEQ ID NO: 36 - protein, 20 aa, Artificial Sequence
  h_Nb5 CDR3
AARLQSATSHSDLREDEFNS

SEQ ID NO: 37 - protein, 120 aa, Artificial Sequence
  h_Nb6 Amino acid sequence of VHH
DVQLQESGGGLAQPGGSLRLSCAASGFTFSSYAMSWARQAPGKGLEWVAGIYRGGSDTYYADSVKGRFTISRDNTKNTLYLQMNSLKPEDTALYYCIQGWGLGYANYDYWGQGTQVTVSS

SEQ ID NO: 38 - protein, 8 aa, Artificial Sequence
  h_Nb6 CDR2
IYRGGSDT

SEQ ID NO: 39 - protein, 13 aa, Artificial Sequence
  h_Nb6 CDR3
IQGWGLGYANYDY

SEQ ID NO: 40 - protein, 116 aa, Artificial Sequence
  h_Nb9 Amino acid sequence of VHH
DVQLQESGGGLVQPGGSLRLSCASSGSIFGLGVKGWYRQPPGNQREMVAQIISGGRISYADSVKGRFTISRDNAKNTVYLQMNSLKPEDTAVYYCNAWGPGQRNYWGRGTQVTVSS

SEQ ID NO: 41 - protein, 8 aa, Artificial Sequence
  h_Nb9 CDR1
GSIFGLGV

SEQ ID NO: 42 - protein, 7 aa, Artificial Sequence
  h_Nb9 CDR2
IISGGRI

SEQ ID NO: 43 - protein, 10 aa, Artificial Sequence
  h_Nb9 CDR3
NAWGPGQRNY

SEQ ID NO: 44 - protein, 127 aa, Artificial Sequence
  h_Nb12 Amino acid sequence of VHH
DVQLQESGGGLVQAGGSLRLSCAASGRTFSSRAMGWFRQAPGKEREFVAAISGSGRNTYYADSVKGRFTISRDNAKNSVNLQMNSLKPEDTAVYYCNAAGGGITIATMTQRTQYDYWGQGTQVTVSS

SEQ ID NO: 45 - protein, 8 aa, Artificial Sequence
  h_Nb12CDR1
GRTFSSRA

SEQ ID NO: 46 - protein, 8 aa, Artificial Sequence
  h_Nb12 CDR2
ISGSGRNT

SEQ ID NO: 47 - protein, 20 aa, Artificial Sequence
  h_Nb12 CDR3
NAAGGGITIATMTQRTQYDY

SEQ ID NO: 48 - protein, 123 aa, Artificial Sequence
  h_Nb13 Amino acid sequence of VHH
DVQLQESGGGLVQPGGSLRLSCAASGSIFSINAMGWYRQAPGKSRELVAAITSGGSTNYADSVKGRFTISRDTAKNTVYLLMNSLEPEDTAVYYCNVERRRPPHYLSEYDFDWGQGTQVTVSS

SEQ ID NO: 49 - protein, 8 aa, Artificial Sequence
  h_Nb13CDR1
GSIFSINA

SEQ ID NO: 50 - protein, 7 aa, Artificial Sequence
  h_Nb13 CDR2,h_Nb26 CDR2
ITSGGST

SEQ ID NO: 51 - protein, 17 aa, Artificial Sequence
  h_Nb13 CDR3
NVERRRPPHYLSEYDFD

SEQ ID NO: 52 - protein, 124 aa, Artificial Sequence
  h_Nb19 Amino acid sequence of VHH
DVQLQESGGGLVQAGGSLRLSCAASGRTFSGYAMAWFRQAPGKEREFVAAISGSGGRTYYADSRFTISRDNAKNTLYLQMNSLKPEDTAGYYCAAAGEGITIATMTQRTQYDYWGQGTQVTVSS

SEQ ID NO: 53 - protein, 8 aa, Artificial Sequence
  h_Nb19CDR1
GRTFSGYA

SEQ ID NO: 54 - protein, 8 aa, Artificial Sequence
  h_Nb19 CDR2
ISGSGGRT

SEQ ID NO: 55 - protein, 20 aa, Artificial Sequence
  h_Nb19 CDR3
AAAGEGITIATMTQRTQYDY

SEQ ID NO: 56 - protein, 123 aa, Artificial Sequence
  h_Nb26 Amino acid sequence of VHH
DVQLQESGGGLVQPGGSLRLSCAAPGSIFRINAMGWYRQAPGKQRELVAAITSGGSTNYADSVQGRFTISRDNAKNTVYLQMNSLKPEDTAVYYCNVERRRPPHYYSDYDFDWGQGTQVTVSS

SEQ ID NO: 57 - protein, 8 aa, Artificial Sequence
  h_Nb26CDR1
GSIFRINA

SEQ ID NO: 58 - protein, 17 aa, Artificial Sequence
  h_Nb26 CDR3
NVERRRPPHYYSDYDFD

SEQ ID NO: 59 - protein, 121 aa, Artificial Sequence
  h_Nb30 Amino acid sequence of VHH
DVQLQESGGGLVQPGESLRVSCAASGFTFSNYYMTWVRQAPGKGLEWVSFLNPSSSERFYADSVKGRFTISRDNAKNTLDLLMHSLKPEDTALYYCARHLKYNWAPNYDYWGQGTQVTVSS

SEQ ID NO: 60 - protein, 8 aa, Artificial Sequence
  h_Nb30CDR1
GFTFSNYY

SEQ ID NO: 61 - protein, 8 aa, Artificial Sequence
  h_Nb30 CDR2
LNPSSSER

SEQ ID NO: 62 - protein, 14 aa, Artificial Sequence
  h_Nb30 CDR3
ARHLKYNWAPNYDY

SEQ ID NO: 63 - protein, 117 aa, Artificial Sequence
  h_Nb1_1
QVQLVESGGGLVQPGGSLRLSCAASGFTFSSYAMSWVRQAPGKGLEWVSAINSGGDNTYYADSVKGRFTISRDNSKNTLYLQMNSLRAEDTAVYYCARGPKLCFSSWGQGTLVTVSS

SEQ ID NO: 64 - protein, 117 aa, Artificial Sequence
  h_Nb1_2
QVQLVESGGGLVQPGGSLRLSCAASGFTFSSYAMSWVRQAPGKGLEWVSDINSGGDNTDYADSVKGRFTISRDNAKNTLYLQMNSLRAEDTAVYYCARGPKLCFSSWGQGTQVTVSS

SEQ ID NO: 65 - protein, 117 aa, Artificial Sequence
  h_Nb1_3
QVQLVESGGGLVQPGGSLRLSCAASGFTFSSYAMSWVRQAPGKGLEWVSDINSGGDNTDYADSVKGRFTISRDNSKNTLYLQMNSLRAEDTAVYYCARGPKLCFSSWGQGTQVTVSS

SEQ ID NO: 66 - protein, 117 aa, Artificial Sequence
  h_Nb1_4
QVQLVESGGGLVQPGGSLRLSCAASGFTFSSYAMSWVRQAPGKGLEWVSDINSGGDNTDYADSVKGRFTISRDNAKNTLYLQMNSLKAEDTAVYYCARGPKLCFSSWGQGTQVTVSS

SEQ ID NO: 67 - protein, 117 aa, Artificial Sequence
  h_Nb1_5
QVQLVESGGGLVQPGGSLRLSCAASGFTFSSYAMSWVRQAPGKGLEWVSDINSGGDNTDYADSVKGRFTISRDNSKNTLYLQMNSLKAEDTAVYYCARGPKLCFSSWGQGTQVTVSS

SEQ ID NO: 68 - protein, 115 aa, Artificial Sequence
  h_Nb2_1
QVQLVESGGGLVQPGGSLRLSCAASGFTFGDRWMYWVRQAPGKGLEWVSAINPAGRSTYYADSVKGRFTISRDNSKNTLYLQMNSLRAEDTAVYYCTKDPGGYQWGQGTLVTVSS

SEQ ID NO: 69 - protein, 115 aa, Artificial Sequence
  h_Nb2_2
QVQLLESGGGLVQPGGSLRLSCAASGFTFGDRWMYWLRQAPGKGLEWVSSINPAGRSTYYADSVKGRFTISRDNSKNTLYLQMNSLRAEDTAVYYCTKDPGGYQKGQGTQVTVSS

SEQ ID NO: 70 - protein, 115 aa, Artificial Sequence
  h_Nb2_3
QVQLVESGGGLVQPGGSLRLSCAASGFTFGDRWMYWLRQAPGKGLEWVSSINPAGRSTYYADSVKGRFTISRDNAKNSLYLQMNSLRAEDTAVYYCTKDPGGYQKGQGTQVTVSS

SEQ ID NO: 71 - protein, 115 aa, Artificial Sequence
  h_Nb2_4
QVQLLESGGGLVQPGGSLRLSCAASGFTFGDRWMYWVRQAPGKGLEWVSSINPAGRSTYYADSVKGRFTISRDNSKNTLYLQMNSLRAEDTAVYYCTKDPGGYQKGQGTQVTVSS

SEQ ID NO: 72 - protein, 115 aa, Artificial Sequence
  h_Nb2_5
QVQLVESGGGLVQPGGSLRLSCAASGFTFGDRWMYWVRQAPGKGLEWVSSINPAGRSTYYADSVKGRFTISRDNAKNSLYLQMNSLRAEDTAVYYCTKDPGGYQKGQGTQVTVSS

SEQ ID NO: 73 - protein, 118 aa, Artificial Sequence
  h_Nb4_1
QVQLVESGGGLVQPGGSLRLSCAASSRMFSGYTMGWVRQAPGKGLEWVSAIANGGFTYYADSVKGRFTISRDNSKNTLYLQMNSLRAEDTAVYYCNLVLVNGIPTRNWGQGTLVTVSS

SEQ ID NO: 74 - protein, 118 aa, Artificial Sequence
  h_Nb4_2
QVQLLESGGGLVQPGGSLRLSCAASSRMFSGYTMGWYRQAPGKGLEWVAQIANGGFTDYIDSVKGRFTISRDNSKNTMYLQMNSLRAEDTAVYYCNLVLVNGIPTRNWGQGTQVTVSS

SEQ ID NO: 75 - protein, 127 aa, Artificial Sequence
  h_Nb5_1
QVQLVESGGGLVQPGGSLRLSCAASGRDLMFYDVAWVRQAPGKGLEWVSAIRSSGTLTYYADSVKGRFTISRDNSKNTLYLQMNSLRAEDTAVYYCAARLQSATSHSDLREDEFNSWGQGTLVTVSS

SEQ ID NO: 76 - protein, 127 aa, Artificial Sequence
  h_Nb5_2
QVQLQESGGGAVQSGESLRLSCAASGRDLMFYDVAWFRQAPGKEREGVSYIRSSGTLTKYADSVKGRFTISRDNDKNTVSLQMNSLNPEDTAKYYCAARLQSATSHSDLREDEFNSWGQGTQVTVSS

SEQ ID NO: 77 - protein, 127 aa, Artificial Sequence
  h_Nb5_3
QVQLVESGGGLVQPGGSLRLSCAASGRDLMFYDVAWVRQAPGKGLEWVSYIRSSGTLTKYADSVKGRFTISRDNSKNTVYLQMNSLRAEDTAVYYCAARLQSATSHSDLREDEFNSWGQGTQVTVSS

SEQ ID NO: 78 - protein, 120 aa, Artificial Sequence
  h_Nb6_1
QVQLVESGGGLVQPGGSLRLSCAASGFTFSSYAMSWVRQAPGKGLEWVSAIYRGGSDTYYADSVKGRFTISRDNSKNTLYLQMNSLRAEDTAVYYCIQGWGLGYANYDYWGQGTLVTVSS

SEQ ID NO: 79 - protein, 120 aa, Artificial Sequence
  h_Nb6_2
QVQLLESGGGLVQPGGSLRLSCAASGFTFSSYAMSWARQAPGKGLEWVAGIYRGGSDTYYADSVKGRFTISRDNSKNTLYLQMNSLRAEDTAVYYCIQGWGLGYANYDYWGQGTQVTVSS

SEQ ID NO: 80 - protein, 114 aa, Artificial Sequence
  h_Nb9_1
QVQLVESGGGLVQPGGSLRLSCAASGSIFGLGVKGWVRQAPGKGLEWVSAIISGGRIYYADSVKGRFTISRDNSKNTLYLQMNSLRAEDTAVYYCNAWGPGQRNYWGQGTLVTV

SEQ ID NO: 81 - protein, 116 aa, Artificial Sequence
  h_Nb9_2
QVQLVESGGGLVQPGGSLRLSCASSGSIFGLGVKGWVRQAPGKGLEWVAQIISGGRISYADSVKGRFTISRDNAKNTVYLQMNSLRAEDTAVYYCNAWGPGQRNYWGRGTQVTVSS

SEQ ID NO: 82 - protein, 127 aa, Artificial Sequence
  h_Nb12_1
QVQLVESGGGLVQPGGSLRLSCAASGRTFSSRAMGWVRQAPGKGLEWVSAISGSGRNTYYADSVKGRFTISRDNSKNTLYLQMNSLRAEDTAVYYCNAAGGGITIATMTQRTQYDYWGQGTLVTVSS

SEQ ID NO: 83 - protein, 127 aa, Artificial Sequence
  h_Nb12_2
QVQLVESGGGLVQPGGSLRLSCAASGRTFSSRAMGWFRQAPGKELEFVAAISGSGRNTYYADSVKGRFTISRDNAKNSVYLQMNSLRAEDTAVYYCNAAGGGITIATMTQRTQYDYWGQGTQVTVSS

SEQ ID NO: 84 - protein, 123 aa, Artificial Sequence
  h_Nb13_1
QVQLVESGGGLVQPGGSLRLSCAASGSIFSINAMGWVRQAPGKGLEWVSAITSGGSTYYADSVKGRFTISRDNSKNTLYLQMNSLRAEDTAVYYCNVERRRPPHYLSEYDFDWGQGTLVTVSS

SEQ ID NO: 85 - protein, 123 aa, Artificial Sequence
  h_Nb13_2
EVQLVESGGGLVQPGGSLRLSCAASGSIFSINAMGWVRQAPGKGLEWVAAITSGGSTNYADSVKGRFTISRDNAKNTVYLQMNSLRAEDTAVYYCNVERRRPPHYLSEYDFDWGQGTQVTVSS

SEQ ID NO: 86 - protein, 124 aa, Artificial Sequence
  h_Nb19_1
QVQLVESGGGLVQPGGSLRLSCAASGRTFSGYAMSWVRQAPGKGLEWVSAISGSGYYADSVKGRFTISRDNSKNTLYLQMNSLRAEDTAVYYCAAAGEGITIATMTQRTQYDYWGQGTLVTVSS

SEQ ID NO: 87 - protein, 124 aa, Artificial Sequence
  h_Nb19_2
QVQLVESGGGLVQPGGSLRLSCAASGRTFSGYAMAWFRQAPGKGREFVAAISGSGGRTYYADSRFTISRDNAKNTLYLQMNSLRAEDTAVYYCAAAGEGITIATMTQRTQYDYWGQGTQVTVSS

SEQ ID NO: 88 - protein, 123 aa, Artificial Sequence
  h_Nb26_1
QVQLVESGGGLVQPGGSLRLSCAASGSIFRINAMGWVRQAPGKGLEWVSAITSGGSTYYADSVKGRFTISRDNSKNTLYLQMNSLRAEDTAVYYCNVERRRPPHYYSDYDFDWGQGTLVTVSS

SEQ ID NO: 89 - protein, 123 aa, Artificial Sequence
  h_Nb26_2
QVQLVQSGAEVKKPGASVKVSCKASGSIFRINAMGWYRQAPGQGLEWVAAITSGGSTNYADSVQGRFTITRDNSTSTVYLELRSLRSDDTAVYYCNVERRRPPHYYSDYDFDWGQGTQVTVSS

SEQ ID NO: 90 - protein, 121 aa, Artificial Sequence
  h_Nb30_1
QVQLVESGGGLVQPGGSLRLSCAASGFTFSNYYMSWVRQAPGKGLEWVSALNPSSSERYYADSVKGRFTISRDNSKNTLYLQMNSLRAEDTAVYYCARHLKYNWAPNYDYWGQGTLVTVSS

SEQ ID NO: 91 - protein, 121 aa, Artificial Sequence
  h_Nb30_2
EVQLVESGGGLVQPGGSLRLSCAASGFTFSNYYMTWVRQAPGKGLEWVSFLNPSSSERFYADSVKGRFTISRDNAKNTLDLQMNSLRAEDTAVYYCARHLKYNWAPNYDYWGQGTQVTVSS

SEQ ID NO: 92 - protein, 117 aa, Artificial Sequence
  h_Nb1_A61N
DVQLQESGGGLVQPGGSLRLSCAASGFTFSSYAMSWVRQAPGKGLEWVSDINSGGDNTDYNDSVKGRFTISRDNAKNTLYLQMNSLKPEDTAVYYCARGPKLCFSSWGQGTQVTVSS

SEQ ID NO: 93 - protein, 117 aa, Artificial Sequence
  h_Nb1_A61Q
DVQLQESGGGLVQPGGSLRLSCAASGFTFSSYAMSWVRQAPGKGLEWVSDINSGGDNTDYQDSVKGRFTISRDNAKNTLYLQMNSLKPEDTAVYYCARGPKLCFSSWGQGTQVTVSS

SEQ ID NO: 94 - protein, 117 aa, Artificial Sequence
  h_Nb1_A61K
DVQLQESGGGLVQPGGSLRLSCAASGFTFSSYAMSWVRQAPGKGLEWVSDINSGGDNTDYKDSVKGRFTISRDNAKNTLYLQMNSLKPEDTAVYYCARGPKLCFSSWGQGTQVTVSS

SEQ ID NO: 95 - protein, 117 aa, Artificial Sequence
  h_Nb1_D59R
DVQLQESGGGLVQPGGSLRLSCAASGFTFSSYAMSWVRQAPGKGLEWVSDINSGGDNTRYADSVKGRFTISRDNAKNTLYLQMNSLKPEDTAVYYCARGPKLCFSSWGQGTQVTVSS

SEQ ID NO: 96 - protein, 117 aa, Artificial Sequence
  h_Nb1_D59M
DVQLQESGGGLVQPGGSLRLSCAASGFTFSSYAMSWVRQAPGKGLEWVSDINSGGDNTMYADSVKGRFTISRDNAKNTLYLQMNSLKPEDTAVYYCARGPKLCFSSWGQGTQVTVSS

SEQ ID NO: 97 - protein, 117 aa, Artificial Sequence
  h_Nb1_D59F
DVQLQESGGGLVQPGGSLRLSCAASGFTFSSYAMSWVRQAPGKGLEWVSDINSGGDNTFYADSVKGRFTISRDNAKNTLYLQMNSLKPEDTAVYYCARGPKLCFSSWGQGTQVTVSS

SEQ ID NO: 98 - protein, 117 aa, Artificial Sequence
  h_Nb1_D62W
DVQLQESGGGLVQPGGSLRLSCAASGFTFSSYAMSWVRQAPGKGLEWVSDINSGGDNTDYAWSVKGRFTISRDNAKNTLYLQMNSLKPEDTAVYYCARGPKLCFSSWGQGTQVTVSS

SEQ ID NO: 99 - protein, 117 aa, Artificial Sequence
  h_Nb1_D62Y
DVQLQESGGGLVQPGGSLRLSCAASGFTFSSYAMSWVRQAPGKGLEWVSDINSGGDNTDYAYSVKGRFTISRDNAKNTLYLQMNSLKPEDTAVYYCARGPKLCFSSWGQGTQVTVSS

SEQ ID NO: 100 - protein, 117 aa, Artificial Sequence
  h_Nb1_C103K
DVQLQESGGGLVQPGGSLRLSCAASGFTFSSYAMSWVRQAPGKGLEWVSDINSGGDNTDYADSVKGRFTISRDNAKNTLYLQMNSLKPEDTAVYYCARGPKLKFSSWGQGTQVTVSS

SEQ ID NO: 101 - protein, 117 aa, Artificial Sequence
  h_Nb1_C103M
DVQLQESGGGLVQPGGSLRLSCAASGFTFSSYAMSWVRQAPGKGLEWVSDINSGGDNTDYADSVKGRFTISRDNAKNTLYLQMNSLKPEDTAVYYCARGPKLMFSSWGQGTQVTVSS

SEQ ID NO: 102 - protein, 117 aa, Artificial Sequence
  h_Nb1_C103W
DVQLQESGGGLVQPGGSLRLSCAASGFTFSSYAMSWVRQAPGKGLEWVSDINSGGDNTDYADSVKGRFTISRDNAKNTLYLQMNSLKPEDTAVYYCARGPKLWFSSWGQGTQVTVSS

SEQ ID NO: 103 - protein, 117 aa, Artificial Sequence
  h_Nb1_G99R
DVQLQESGGGLVQPGGSLRLSCAASGFTFSSYAMSWVRQAPGKGLEWVSDINSGGDNTDYADSVKGRFTISRDNAKNTLYLQMNSLKPEDTAVYYCARRPKLCFSSWGQGTQVTVSS

SEQ ID NO: 104 - protein, 117 aa, Artificial Sequence
  h_Nb1_G99Q
DVQLQESGGGLVQPGGSLRLSCAASGFTFSSYAMSWVRQAPGKGLEWVSDINSGGDNTDYADSVKGRFTISRDNAKNTLYLQMNSLKPEDTAVYYCARQPKLCFSSWGQGTQVTVSS

SEQ ID NO: 105 - protein, 117 aa, Artificial Sequence
  h_Nb1_G99W
DVQLQESGGGLVQPGGSLRLSCAASGFTFSSYAMSWVRQAPGKGLEWVSDINSGGDNTDYADSVKGRFTISRDNAKNTLYLQMNSLKPEDTAVYYCARWPKLCFSSWGQGTQVTVSS

SEQ ID NO: 106 - protein, 117 aa, Artificial Sequence
  h_Nb1_G99Y
DVQLQESGGGLVQPGGSLRLSCAASGFTFSSYAMSWVRQAPGKGLEWVSDINSGGDNTDYADSVKGRFTISRDNAKNTLYLQMNSLKPEDTAVYYCARYPKLCFSSWGQGTQVTVSS

SEQ ID NO: 107 - protein, 115 aa, Artificial Sequence
  h_Nb2_G30R
DVQLQESGGGLVQPGGSLRLSCAASGFTFRDRWMYWLRQAPGKGLEWVSSINPAGRSTYYADSVKGRFTISRDNAKNTLYLQMNSLKSEDTAVYYCTKDPGGYQKGQGTQVTVSS

SEQ ID NO: 108 - protein, 115 aa, Artificial Sequence
  h_Nb2_G30F
DVQLQESGGGLVQPGGSLRLSCAASGFTFFDRWMYWLRQAPGKGLEWVSSINPAGRSTYYADSVKGRFTISRDNAKNTLYLQMNSLKSEDTAVYYCTKDPGGYQKGQGTQVTVSS

SEQ ID NO: 109 - protein, 115 aa, Artificial Sequence
  h_Nb2_G30W
DVQLQESGGGLVQPGGSLRLSCAASGFTFWDRWMYWLRQAPGKGLEWVSSINPAGRSTYYADSVKGRFTISRDNAKNTLYLQMNSLKSEDTAVYYCTKDPGGYQKGQGTQVTVSS

SEQ ID NO: 110 - protein, 115 aa, Artificial Sequence
  h_Nb2_G101R
DVQLQESGGGLVQPGGSLRLSCAASGFTFGDRWMYWLRQAPGKGLEWVSSINPAGRSTYYADSVKGRFTISRDNAKNTLYLQMNSLKSEDTAVYYCTKDPRGYQKGQGTQVTVSS

SEQ ID NO: 111 - protein, 115 aa, Artificial Sequence
  h_Nb2_G101W
DVQLQESGGGLVQPGGSLRLSCAASGFTFGDRWMYWLRQAPGKGLEWVSSINPAGRSTYYADSVKGRFTISRDNAKNTLYLQMNSLKSEDTAVYYCTKDPWGYQKGQGTQVTVSS

SEQ ID NO: 112 - protein, 115 aa, Artificial Sequence
  h_Nb2_G101Y
DVQLQESGGGLVQPGGSLRLSCAASGFTFGDRWMYWLRQAPGKGLEWVSSINPAGRSTYYADSVKGRFTISRDNAKNTLYLQMNSLKSEDTAVYYCTKDPGYYQKGQGTQVTVSS

SEQ ID NO: 113 - protein, 115 aa, Artificial Sequence
  h_Nb2_F29R
DVQLQESGGGLVQPGGSLRLSCAASGFTRGDRWMYWLRQAPGKGLEWVSSINPAGRSTYYADSVKGRFTISRDNAKNTLYLQMNSLKSEDTAVYYCTKDPGGYQKGQGTQVTVSS

SEQ ID NO: 114 - protein, 115 aa, Artificial Sequence
  h_Nb2_F29W
DVQLQESGGGLVQPGGSLRLSCAASGFTWGDRWMYWLRQAPGKGLEWVSSINPAGRSTYYADSVKGRFTISRDNAKNTLYLQMNSLKSEDTAVYYCTKDPGGYQKGQGTQVTVSS

SEQ ID NO: 115 - protein, 115 aa, Artificial Sequence
  h_Nb2_P100R
DVQLQESGGGLVQPGGSLRLSCAASGFTFGDRWMYWLRQAPGKGLEWVSSINPAGRSTYYADSVKGRFTISRDNAKNTLYLQMNSLKSEDTAVYYCTKDRGGYQKGQGTQVTVSS

SEQ ID NO: 116 - protein, 115 aa, Artificial Sequence
  h_Nb2_P100Q
DVQLQESGGGLVQPGGSLRLSCAASGFTFGDRWMYWLRQAPGKGLEWVSSINPAGRSTYYADSVKGRFTISRDNAKNTLYLQMNSLKSEDTAVYYCTKDQGGYQKGQGTQVTVSS

SEQ ID NO: 117 - protein, 115 aa, Artificial Sequence
  h_Nb2_P100E
DVQLQESGGGLVQPGGSLRLSCAASGFTFGDRWMYWLRQAPGKGLEWVSSINPAGRSTYYADSVKGRFTISRDNAKNTLYLQMNSLKSEDTAVYYCTKDEGGYQKGQGTQVTVSS